European Patent Application EP 4 275 688 A2, published November 15, 2023. Title: METHOD OF AMELIORATING OR PREVENTING THE WORSENING OR THE PROGRESSION OF SYMPTOMS OF BPH. Applicant: Nymox Corporation. Application EP EP17764662, filed August 29, 2017. The sequence listing filed with the application follows.

SEQUENCE LISTING (118 sequences)

SEQ ID NO: 1 - protein, 15 aa, synthetic construct
  REGION 1..15: note = Description of Artificial Sequence: Synthetic peptide
MEFSLLLPRLECNGA

SEQ ID NO: 2 - protein, 15 aa, synthetic construct
  REGION 1..15: note = Description of Artificial Sequence: Synthetic peptide
GAISAHRNLRLPGSS

SEQ ID NO: 3 - protein, 17 aa, synthetic construct
  REGION 1..17: note = Description of Artificial Sequence: Synthetic peptide
DSPASASPVAGITGMCT

SEQ ID NO: 4 - protein, 16 aa, synthetic construct
  REGION 1..16: note = Description of Artificial Sequence: Synthetic peptide
MCTHARLILYFFLVEM

SEQ ID NO: 5 - protein, 11 aa, synthetic construct
  REGION 1..11: note = Description of Artificial Sequence: Synthetic peptide
YFFLVEMEFLH

SEQ ID NO: 6 - protein, 11 aa, synthetic construct
  REGION 1..11: note = Description of Artificial Sequence: Synthetic peptide
VGQAGLELPTS

SEQ ID NO: 7 - protein, 17 aa, synthetic construct
  REGION 1..17: note = Description of Artificial Sequence: Synthetic peptide
DDPSVSASQSARYRTGH

SEQ ID NO: 8 - protein, 14 aa, synthetic construct
  REGION 1..14: note = Description of Artificial Sequence: Synthetic peptide
TGHHARLCLANFCG

SEQ ID NO: 9 - protein, 17 aa, synthetic construct
  REGION 1..17: note = Description of Artificial Sequence: Synthetic peptide
ANFCGRNRVSLMCPSWS

SEQ ID NO: 10 - protein, 19 aa, synthetic construct
  REGION 1..19: note = Description of Artificial Sequence: Synthetic peptide
PELKQSTCLSLPKCWDYRR

SEQ ID NO: 11 - protein, 17 aa, synthetic construct
  REGION 1..17: note = Description of Artificial Sequence: Synthetic peptide
LKQSTCLSLPKCWDYRR

SEQ ID NO: 12 - protein, 14 aa, synthetic construct
  REGION 1..14: note = Description of Artificial Sequence: Synthetic peptide
STCLSLPKCWDYRR

SEQ ID NO: 13 - protein, 11 aa, synthetic construct
  REGION 1..11: note = Description of Artificial Sequence: Synthetic peptide
LSLPKCWDYRR

SEQ ID NO: 14 - protein, 13 aa, synthetic construct
  REGION 1..13: note = Description of Artificial Sequence: Synthetic peptide
KCWDYRRAAVPGL

SEQ ID NO: 15 - protein, 19 aa, synthetic construct
  REGION 1..19: note = Description of Artificial Sequence: Synthetic peptide
KCWDYRRAAVPGLFILFFL

SEQ ID NO: 16 - protein, 24 aa, synthetic construct
  REGION 1..24: note = Description of Artificial Sequence: Synthetic peptide
KCWDYRRAAVPGLFILFFLRHRCP

SEQ ID NO: 17 - protein, 38 aa, synthetic construct
  REGION 1..38: note = Description of Artificial Sequence: Synthetic polypeptide
KCWDYRRAAVPGLFILFFLRHRCPTLTQDEVQWCDHSS

SEQ ID NO: 18 - protein, 5 aa, synthetic construct
  REGION 1..5: note = Description of Artificial Sequence: Synthetic peptide
WDYRR

SEQ ID NO: 19 - protein, 13 aa, synthetic construct
  REGION 1..13: note = Description of Artificial Sequence: Synthetic peptide
FILFFLRHRCPTL

SEQ ID NO: 20 - protein, 25 aa, synthetic construct
  REGION 1..25: note = Description of Artificial Sequence: Synthetic peptide
FILFFLRHRCPTLTQDEVQWCDHSS

SEQ ID NO: 21 - protein, 29 aa, synthetic construct
  REGION 1..29: note = Description of Artificial Sequence: Synthetic peptide
HRCPTLTQDEVQWCDHSSLQPSTPEIKHP

SEQ ID NO: 22 - protein, 14 aa, synthetic construct
  REGION 1..14: note = Description of Artificial Sequence: Synthetic peptide
PASASQVAGTKDMH

SEQ ID NO: 23 - protein, 18 aa, synthetic construct
  REGION 1..18: note = Description of Artificial Sequence: Synthetic peptide
DMHHYTWLIFIFIFNFLR

SEQ ID NO: 24 - protein, 19 aa, synthetic construct [sequence omitted]

SEQ ID NO: 25 - protein, 45 aa, synthetic construct
  REGION 1..45: note = Description of Artificial Sequence: Synthetic polypeptide
SVTQAGVQWRNLGSLQPLPPGFKLFSCPSLLSSWDYRRPPRLANF

SEQ ID NO: 26 - protein, 19 aa, synthetic construct
  REGION 1..19: note = Description of Artificial Sequence: Synthetic peptide
PGFKLFSCPSLLSSWDYRR

SEQ ID NO: 27 - protein, 24 aa, synthetic construct
  REGION 1..24: note = Description of Artificial Sequence: Synthetic peptide
FKLFSCPSLLSSWDYRRPPRLANF

SEQ ID NO: 28 - protein, 14 aa, synthetic construct
  REGION 1..14: note = Description of Artificial Sequence: Synthetic peptide
FSCPSLLSSWDYRR

SEQ ID NO: 29 - protein, 10 aa, synthetic construct
  REGION 1..10: note = Description of Artificial Sequence: Synthetic peptide
SLLSSWDYRR

SEQ ID NO: 30 - protein, 5 aa, synthetic construct
  REGION 1..5: note = Description of Artificial Sequence: Synthetic peptide
SSWDY

SEQ ID NO: 31 - protein, 7 aa, synthetic construct
  REGION 1..7: note = Description of Artificial Sequence: Synthetic peptide
SSWDYRR

SEQ ID NO: 32 - protein, 25 aa, synthetic construct
  REGION 1..25: note = Description of Artificial Sequence: Synthetic peptide
SSWDYRRPPRLANFFVFLVEMGFTM

SEQ ID NO: 33 - protein, 11 aa, synthetic construct
  REGION 1..11: note = Description of Artificial Sequence: Synthetic peptide
FVFLVEMGFTM

SEQ ID NO: 34 - protein, 23 aa, synthetic construct
  REGION 1..23: note = Description of Artificial Sequence: Synthetic peptide
MGFTMFARLILISGPCDLPASAS

SEQ ID NO: 35 - protein, 5 aa, synthetic construct
  REGION 1..5: note = Description of Artificial Sequence: Synthetic peptide
ISGPC

SEQ ID NO: 36 - protein, 17 aa, synthetic construct
  REGION 1..17: note = Description of Artificial Sequence: Synthetic peptide
DLPASASQSAGITGVSH

SEQ ID NO: 37 - protein, 17 aa, synthetic construct
  REGION 1..17: note = Description of Artificial Sequence: Synthetic peptide
GVSHHARLIFNFCLFEM

SEQ ID NO: 38 - protein, 10 aa, synthetic construct
  REGION 1..10: note = Description of Artificial Sequence: Synthetic peptide
NFCLFEMESH

SEQ ID NO: 39 - protein, 46 aa, synthetic construct
  REGION 1..46: note = Description of Artificial Sequence: Synthetic polypeptide
SVTQAGVQWPNLGSLQPLPPGLKRFSCLSLPSSWDYGHLPPHPANF

SEQ ID NO: 40 - protein, 19 aa, synthetic construct
  REGION 1..19: note = Description of Artificial Sequence: Synthetic peptide
PPGLKRFSCLSLPSSWDYG

SEQ ID NO: 41 - protein, 14 aa, synthetic construct
  REGION 1..14: note = Description of Artificial Sequence: Synthetic peptide
FSCLSLPSSWDYGH

SEQ ID NO: 42 - protein, 9 aa, synthetic construct
  REGION 1..9: note = Description of Artificial Sequence: Synthetic peptide
LSLPSSWDY

SEQ ID NO: 43 - protein, 37 aa, synthetic construct
  REGION 1..37: note = Description of Artificial Sequence: Synthetic polypeptide
SSWDYGHLPPHPANFCIFIRGGVSPYLSGWSQTPDLR

SEQ ID NO: 44 - protein, 20 aa, synthetic construct
  REGION 1..20: note = Description of Artificial Sequence: Synthetic peptide
PGFFKLFSCPSLLSSWDYRR

SEQ ID NO: 45 - protein, 19 aa, synthetic construct
  REGION 1..19: note = Description of Artificial Sequence: Synthetic peptide
PELKQSTCLSLPKCWDYRR

SEQ ID NO: 46 - protein, 19 aa, synthetic construct
  REGION 1..19: note = Description of Artificial Sequence: Synthetic peptide
PPGLKRFSCLSLPSSWDYG

SEQ ID NO: 47 - protein, 14 aa, synthetic construct
  REGION 1..14: note = Description of Artificial Sequence: Synthetic peptide
FSCLSLPSSWDYGH

SEQ ID NO: 48 - protein, 14 aa, synthetic construct
  REGION 1..14: note = Description of Artificial Sequence: Synthetic peptide
STCLSLPKCWDYRR

SEQ ID NO: 49 - protein, 14 aa, synthetic construct
  REGION 1..14: note = Description of Artificial Sequence: Synthetic peptide
FSCPSLLSSWDYRR

SEQ ID NO: 50 - protein, 9 aa, synthetic construct
  REGION 1..9: note = Description of Artificial Sequence: Synthetic peptide
LSLPSSWDY

SEQ ID NO: 51 - protein, 11 aa, synthetic construct
  REGION 1..11: note = Description of Artificial Sequence: Synthetic peptide
LSLPKCWDYRR

SEQ ID NO: 52 - protein, 10 aa, synthetic construct
  REGION 1..10: note = Description of Artificial Sequence: Synthetic peptide
SLLSSWDYRR

SEQ ID NO: 53 - protein, 9 aa, synthetic construct
  REGION 1..9: note = Description of Artificial Sequence: Synthetic peptide
LPSSWDYRR

SEQ ID NO: 54 - protein, 7 aa, synthetic construct
  REGION 1..7: note = Description of Artificial Sequence: Synthetic peptide
SSWDYRR

SEQ ID NO: 55 - protein, 5 aa, synthetic construct
  REGION 1..5: note = Description of Artificial Sequence: Synthetic peptide
SSWDY

SEQ ID NO: 56 - protein, 13 aa, synthetic construct
  REGION 1..13: note = Description of Artificial Sequence: Synthetic peptide
SSWDYRRFILFFL

SEQ ID NO: 57 - protein, 11 aa, synthetic construct
  REGION 1..11: note = Description of Artificial Sequence: Synthetic peptide
WDYRRFIFNFL

SEQ ID NO: 58 - protein, 6 aa, synthetic construct
  REGION 1..6: note = Description of Artificial Sequence: Synthetic peptide
FNFCLF

SEQ ID NO: 59 - protein, 6 aa, synthetic construct
  REGION 1..6: note = Description of Artificial Sequence: Synthetic peptide
FIFNFL

SEQ ID NO: 60 - protein, 13 aa, synthetic construct
  REGION 1..13: note = Description of Artificial Sequence: Synthetic peptide
PASASPVAGITGM

SEQ ID NO: 61 - protein, 13 aa, synthetic construct
  REGION 1..13: note = Description of Artificial Sequence: Synthetic peptide
PASASQVAGTKDM

SEQ ID NO: 62 - protein, 13 aa, synthetic construct
  REGION 1..13: note = Description of Artificial Sequence: Synthetic peptide
PASASQSAGITGV

SEQ ID NO: 63 - protein, 9 aa, synthetic construct
  REGION 1..9: note = Description of Artificial Sequence: Synthetic peptide
PASASPVAG

SEQ ID NO: 64 - protein, 6 aa, synthetic construct
  REGION 1..6: note = Description of Artificial Sequence: Synthetic peptide
FFLVEM

SEQ ID NO: 65 - protein, 9 aa, synthetic construct
  REGION 1..9: note = Description of Artificial Sequence: Synthetic peptide
SVTQAGVQW

SEQ ID NO: 66 - protein, 17 aa, synthetic construct
  REGION 1..17: note = Description of Artificial Sequence: Synthetic peptide
IDQQVLSRIKLEIKRCL

SEQ ID NO: 67 - protein, 9 aa, synthetic construct
  REGION 1..9: note = Description of Artificial Sequence: Synthetic peptide
LSRIKLEIK

SEQ ID NO: 68 - protein, 22 aa, synthetic construct
  REGION 1..22: note = Description of Artificial Sequence: Synthetic peptide
GDHGRPNLSRLKLAIKYEVKKM

SEQ ID NO: 69 - protein, 16 aa, synthetic construct
  REGION 1..16: note = Description of Artificial Sequence: Synthetic peptide
QQSIAVKFLAVFGVSI

SEQ ID NO: 70 - protein, 21 aa, synthetic construct
  REGION 1..21: note = Description of Artificial Sequence: Synthetic peptide
GLLFPVFSVCYLIAPKSPLGL

SEQ ID NO: 71 - protein, 15 aa, synthetic construct
  REGION 1..15: note = Description of Artificial Sequence: Synthetic peptide
MMVCWNRFGKWVYFI

SEQ ID NO: 72 - protein, 15 aa, synthetic construct
  REGION 1..15: note = Description of Artificial Sequence: Synthetic peptide
SAIFNFGPRYLYHGV

SEQ ID NO: 73 - protein, 15 aa, synthetic construct
  REGION 1..15: note = Description of Artificial Sequence: Synthetic peptide
PFYFLILVRIISFLI

SEQ ID NO: 74 - protein, 15 aa, synthetic construct
  REGION 1..15: note = Description of Artificial Sequence: Synthetic peptide
GDMEDVLLNCTLLKR

SEQ ID NO: 75 - protein, 15 aa, synthetic construct
  REGION 1..15: note = Description of Artificial Sequence: Synthetic peptide
SSRFRFWGALVCSMD

SEQ ID NO: 76 - protein, 15 aa, synthetic construct
  REGION 1..15: note = Description of Artificial Sequence: Synthetic peptide
SCRFSRVAVTYRFIT

SEQ ID NO: 77 - protein, 15 aa, synthetic construct
  REGION 1..15: note = Description of Artificial Sequence: Synthetic peptide
LLNIPSPAVWMARNT

SEQ ID NO: 78 - protein, 15 aa, synthetic construct
  REGION 1..15: note = Description of Artificial Sequence: Synthetic peptide
MAQSRLTATSASRVQ

SEQ ID NO: 79 - protein, 15 aa, synthetic construct
  REGION 1..15: note = Description of Artificial Sequence: Synthetic peptide
AILLSQPPKQLGLRA

SEQ ID NO: 80 - protein, 15 aa, synthetic construct
  REGION 1..15: note = Description of Artificial Sequence: Synthetic peptide
PANTPLIFVFSLEAG

SEQ ID NO: 81 - protein, 15 aa, synthetic construct
  REGION 1..15: note = Description of Artificial Sequence: Synthetic peptide
FHHICQAGLKLLTSG

SEQ ID NO: 82 - protein, 15 aa, synthetic construct
  REGION 1..15: note = Description of Artificial Sequence: Synthetic peptide
DPPASAFQSAGITGV

SEQ ID NO: 83 - protein, 15 aa, synthetic construct
  REGION 1..15: note = Description of Artificial Sequence: Synthetic peptide
SHLTQPANLDKKICS

SEQ ID NO: 84 - protein, 22 aa, synthetic construct
  REGION 1..22: note = Description of Artificial Sequence: Synthetic peptide
NGGSCYVAQAGLKLLASCNPSK

SEQ ID NO: 85 - protein, 15 aa, synthetic construct
  REGION 1..15: note = Description of Artificial Sequence: Synthetic peptide
MWTLKSSLVLLLCLT

SEQ ID NO: 86 - protein, 15 aa, synthetic construct
  REGION 1..15: note = Description of Artificial Sequence: Synthetic peptide
CSYAFMFSSLRQKTS

SEQ ID NO: 87 - protein, 15 aa, synthetic construct
  REGION 1..15: note = Description of Artificial Sequence: Synthetic peptide
EPQGKVPCGEHFRIR

SEQ ID NO: 88 - protein, 15 aa, synthetic construct
  REGION 1..15: note = Description of Artificial Sequence: Synthetic peptide
QNLPEHTQGWLGSKW

SEQ ID NO: 89 - protein, 15 aa, synthetic construct
  REGION 1..15: note = Description of Artificial Sequence: Synthetic peptide
LWLLFAVVPFVILKC

SEQ ID NO: 90 - protein, 15 aa, synthetic construct
  REGION 1..15: note = Description of Artificial Sequence: Synthetic peptide
QRDSEKNKVRMAPFF

SEQ ID NO: 91 - protein, 16 aa, synthetic construct
  REGION 1..16: note = Description of Artificial Sequence: Synthetic peptide
LHHIDSISGVSGKRMF

SEQ ID NO: 92 - protein, 15 aa, synthetic construct
  REGION 1..15: note = Description of Artificial Sequence: Synthetic peptide
EAYYTMLHLPTTNRP

SEQ ID NO: 93 - protein, 15 aa, synthetic construct
  REGION 1..15: note = Description of Artificial Sequence: Synthetic peptide
KIAHCILFNQPHSPR

SEQ ID NO: 94 - protein, 15 aa, synthetic construct
  REGION 1..15: note = Description of Artificial Sequence: Synthetic peptide
SNSHSHPNPLKLHRR

SEQ ID NO: 95 - protein, 15 aa, synthetic construct
  REGION 1..15: note = Description of Artificial Sequence: Synthetic peptide
SHSHNRPRAYILITI

SEQ ID NO: 96 - protein, 15 aa, synthetic construct
  REGION 1..15: note = Description of Artificial Sequence: Synthetic peptide
LPSKLKLRTHSQSHH

SEQ ID NO: 97 - protein, 23 aa, synthetic construct
  REGION 1..23: note = Description of Artificial Sequence: Synthetic peptide
NPLSRTSNSTPTNSFLMTSSKPR

SEQ ID NO: 98 - protein, 15 aa, synthetic construct
  REGION 1..15: note = Description of Artificial Sequence: Synthetic peptide
SSSLGLPKCWDYRHE

SEQ ID NO: 99 - protein, 15 aa, synthetic construct
  REGION 1..15: note = Description of Artificial Sequence: Synthetic peptide
LLSLALMINFRVMAC

SEQ ID NO: 100 - protein, 15 aa, synthetic construct
  REGION 1..15: note = Description of Artificial Sequence: Synthetic peptide
TFKQHIELRQKISIV

SEQ ID NO: 101 - protein, 15 aa, synthetic construct
  REGION 1..15: note = Description of Artificial Sequence: Synthetic peptide
PRKLCCMGPVCPVKI

SEQ ID NO: 102 - protein, 15 aa, synthetic construct
  REGION 1..15: note = Description of Artificial Sequence: Synthetic peptide
ALLTINGHCTWLPAS

SEQ ID NO: 103 - protein, 15 aa, synthetic construct
  REGION 1..15: note = Description of Artificial Sequence: Synthetic peptide
MFVFCLILNREKIKG

SEQ ID NO: 104 - protein, 15 aa, synthetic construct
  REGION 1..15: note = Description of Artificial Sequence: Synthetic peptide
GNSSFFLLSFFFSFQ

SEQ ID NO: 105 - protein, 15 aa, synthetic construct
  REGION 1..15: note = Description of Artificial Sequence: Synthetic peptide
NCCQCFQCRTTEGYA

SEQ ID NO: 106 - protein, 23 aa, synthetic construct
  REGION 1..23: note = Description of Artificial Sequence: Synthetic peptide
VECFYCLVDKAAFECWWFYSFDT

SEQ ID NO: 107 - protein, 15 aa, synthetic construct
  REGION 1..15: note = Description of Artificial Sequence: Synthetic peptide
MEPHTVAQAGVPQHD

SEQ ID NO: 108 - protein, 15 aa, synthetic construct
  REGION 1..15: note = Description of Artificial Sequence: Synthetic peptide
LGSLQSLLPRFKRFS

SEQ ID NO: 109 - protein, 15 aa, synthetic construct
  REGION 1..15: note = Description of Artificial Sequence: Synthetic peptide
CLILPKIWDYRNMNT

SEQ ID NO: 110 - protein, 16 aa, synthetic construct
  REGION 1..16: note = Description of Artificial Sequence: Synthetic peptide
ALIKRNRYTPETGRKS

SEQ ID NO: 111 - protein, 9 aa, synthetic construct
  REGION 1..9: note = Description of Artificial Sequence: Synthetic peptide
IDQQVLSRI

SEQ ID NO: 112 - protein, 8 aa, synthetic construct
  REGION 1..8: note = Description of Artificial Sequence: Synthetic peptide
KLEIKRCL

SEQ ID NO: 113 - protein, 6 aa, synthetic construct
  REGION 1..6: note = Description of Artificial Sequence: Synthetic peptide
VLSRIK

SEQ ID NO: 114 - protein, 7 aa, synthetic construct
  REGION 1..7: note = Description of Artificial Sequence: Synthetic peptide
RIKLEIK

SEQ ID NO: 115 - protein, 13 aa, synthetic construct
  REGION 1..13: note = Description of Artificial Sequence: Synthetic peptide
VLSRIKLEIKRCL

SEQ ID NO: 116 - protein, 13 aa, synthetic construct
  REGION 1..13: note = Description of Artificial Sequence: Synthetic peptide
IDQQVLSRIKLEI

SEQ ID NO: 117 - protein, 5 aa, synthetic construct
  REGION 1..5: note = Description of Artificial Sequence: Synthetic peptide
ETESH

SEQ ID NO: 118 - protein, 6 aa, synthetic construct
  REGION 1..6: note = Description of Artificial Sequence: Synthetic 6xHis tag
HHHHHH